European Patent Specification EP 3 898 992 B1, published May 24, 2023. Title: Hybrid promoters and their uses in therapy, notably for treating type II collagenopathies. Applicant: INSTITUT NATIONAL DE LA SANTE ET DE LA RECHERCHE MEDICALE (INSERM) et al. The sequence listing filed with the application follows.

SEQUENCE LISTING (30 sequences)

SEQ ID NO: 1 - DNA, 716 bp, Homo sapiens
accggtgctaaaagataggtcggggtaacccttcagatctggctcagctagcctgtctccaagatttaggactctgaatctctgtgggctcctccctgtccccactcccaaacgcctgacgcggtgccccctcgccctccgctgctcctttctaccgctttccctcctccctcccatgtcttttccgtccttggtctagggctctcggcctgcgcctctgcaaacaccccctcccctccaactccggcagaactccgaggggaggggccggaggccacccttcccgcctgtggtcagaggggggcagcgccgcagccccgggtttggggggcaggggccatctctgcgccccgcccgatcaggccactcggcgcactaggggtggagggcgggaagcgtgactcccagagaggggggtccggcttgggcaggtgcgggcactggcagggcccaggcgggctccgggggcgggcggttcaggttacagcccagcggggggcagggggcggcccgcggtttgggcgagttcgccagcctcgaaaggggccgggcgcatataacgggcgccgcggcggggagaagacgcagagcgctgctgggctgccgggtctcccgcttccccctcctgctccaagggcctcctgcatgagggcgcggtagagacccggacccgcgccgtgctcctgccgtttcgctgcgctccgcccgatttaaat

SEQ ID NO: 2 - DNA, 77 bp, Homo sapiens
gcgcggggtaaactgggaaagtgatgtcgtgtactggctccgcctttttcccgagggtgggggagaaccgtatataa

SEQ ID NO: 3 - skipped

SEQ ID NO: 4 - DNA, 60 bp, Homo sapiens
ccgagggtgggggagaaccgtatataagtgcagtagtcgccgtgaacgttctttttcgca

SEQ ID NO: 5 - DNA, 1184 bp, Homo sapiens
gaattggctccggtgcccgtcagtgggcagagcgcacatcgcccacagtccccgagaagttggggggaggggtcggcaattgaaccggtgcctagagaaggtggcgcggggtaaactgggaaagtgatgtcgtgtactggctccgcctttttcccgagggtgggggagaaccgtatataagtgcagtagtcgccgtgaacgttctttttcgcaacgggtttgccgccagaacacaggtaagtgccgtgtgtggttcccgcgggcctggcctctttacgggttatggcccttgcgtgccttgaattacttccacctggctgcagtacgtgattcttgatcccgagcttcgggttggaagtgggtgggagagttcgaggccttgcgcttaaggagccccttcgcctcgtgcttgagttgaggcctggcctgggcgctggggccgccgcgtgcgaatctggtggcaccttcgcgcctgtctcgctgctttcgataagtctctagccatttaaaatttttgatgacctgctgcgacgctttttttctggcaagatagtcttgtaaatgcgggccaagatctgcacactggtatttcggtttttggggccgcgggcggcgacggggcccgtgcgtcccagcgcacatgttcggcgaggcggggcctgcgagcgcggccaccgagaatcggacgggggtagtctcaagctggccggcctgctctggtgcctggcctcgcgccgccgtgtatcgccccgccctgggcggcaaggctggcccggtcggcaccagttgcgtgagcggaaagatggccgcttcccggccctgctgcagggagctcaaaatggaggacgcggcgctcgggagagcgggcgggtgagtcacccacacaaaggaaaagggcctttccgtcctcagccgtcgcttcatgtgactccacggagtaccgggcgccgtccaggcacctcgattagttctcgagcttttggagtacgtcgtctttaggttggggggaggggttttatgcgatggagtttccccacactgagtgggtggagactgaagttaggccagcttggcacttgatgtaattctccttggaatttgccctttttgagtttggatcttggttcattctcaagcctcagacagtggttcaaagtttttttcttccatttcaggtgtcgtga

SEQ ID NO: 6 - DNA, 295 bp, Homo sapiens
accccctcccctccaactccggcagaactccgaggggaggggccggaggccacccttcccgcctgtggtcagaggggggcagcgccgcagccccgggtttggggggcaggggccatctctgcgccccgcccgatcaggccactcggcgcactaggggtggagggcgggaagcgtgactcccagagaggggggtccggcttgggcaggtgcgggcactggcagggcccaggcgggctccgggggcgggcggttcaggttacagcccagcggggggcagggggcggcccgcggtttg

SEQ ID NO: 7 - DNA, 40 bp, Homo sapiens
gggcactggcagggcccaggcgggctccgggggcgggcgg

SEQ ID NO: 8 - DNA, 10 bp, Homo sapiens
gggctgccgg

SEQ ID NO: 9 - DNA, 20 bp, Homo sapiens
gcgcggggtaaactgggaaa

SEQ ID NO: 10 - DNA, 20 bp, Homo sapiens
gtactggctccgcctttttc

SEQ ID NO: 11 - DNA, 769 bp, Artificial Sequence
  Hybrid promoter 13a
accggtgctaaaagataggtcggggtaacccttcagatctggctcagctagcctgtctccaagatttaggactctgaatctctgtgggctcctccctgtccccactcccaaacgcctgacgcggtgccccctcgccctccgctgctcctttctaccgctttccctcctccctcccatgtcttttccgtccttggtctagggctctcggcctgcgcctctgcaaacaccccctcccctccaactccggcagaactccgaggggaggggccggaggccacccttcccgcctgtggtcagaggggggcagcgccgcagccccgggtttggggggcaggggccatctctgcgccccgcccgatcaggccactcggcgcactaggggtggagggcgggaagcgtgactcccagagaggggggtccggcttgggcaggtgcgggcactggcagggcccaggcgggctccgggggcgggcggttcaggttacagcccagcggggggcagggggcggcccgcggtttgggcgagttcgccagcctcgagcgcggggtaaactgggaaagtgatgtcgtgtactggctccgcctttttcccgagggtgggggagaaccgtatataacgggcgccgcggcggggagaagacgcagagcgctgctgtctcccgcttccccctcctgctccaagggcctcctgcatgagggcgcggtagagacccggacccgcgccgtgctcctgccgtttcgctgcgctccgcccgatttaaatggatcc

SEQ ID NO: 12 - DNA, 779 bp, Artificial Sequence
  Hybrid promoter 13b
accggtgctaaaagataggtcggggtaacccttcagatctggctcagctagcctgtctccaagatttaggactctgaatctctgtgggctcctccctgtccccactcccaaacgcctgacgcggtgccccctcgccctccgctgctcctttctaccgctttccctcctccctcccatgtcttttccgtccttggtctagggctctcggcctgcgcctctgcaaacaccccctcccctccaactccggcagaactccgaggggaggggccggaggccacccttcccgcctgtggtcagaggggggcagcgccgcagccccgggtttggggggcaggggccatctctgcgccccgcccgatcaggccactcggcgcactaggggtggagggcgggaagcgtgactcccagagaggggggtccggcttgggcaggtgcgggcactggcagggcccaggcgggctccgggggcgggcggttcaggttacagcccagcggggggcagggggcggcccgcggtttgggcgagttcgccagcctcgagcgcggggtaaactgggaaagtgatgtcgtgtactggctccgcctttttcccgagggtgggggagaaccgtatataacgggcgccgcggcggggagaagacgcagagcgctgctgggctgccgggtctcccgcttccccctcctgctccaagggcctcctgcatgagggcgcggtagagacccggacccgcgccgtgctcctgccgtttcgctgcgctccgcccgatttaaatggatcc

SEQ ID NO: 13 - DNA, 713 bp, Artificial Sequence
  Hybrid promoter 14a
accggtgctaaaagataggtcggggtaacccttcagatctggctcagctagcctgtctccaagatttaggactctgaatctctgtgggctcctccctgtccccactcccaaacgcctgacgcggtgccccctcgccctccgctgctcctttctaccgctttccctcctccctcccatgtcttttccgtccttggtctagggctctcggcctgcgcctctgcaaacaccccctcccctccaactccggcagaactccgaggggaggggccggaggccacccttcccgcctgtggtcagaggggggcagcgccgcagccccgggtttggggggcaggggccatctctgcgccccgcccgatcaggccactcggcgcactaggggtggagggcgggaagcgtgactcccagagaggggggtccggcttgggcaggtgcgggcactggcagggcccaggcgggctccgggggcgggcggttcaggttacagcccagcggggggcagggggcggcccgcggtttgggcgagttcgccagcctcgaaaggggccgggcgctatataacgggcgccgcggcggggagaagacgcagagcgctgctgtctcccgcttccccctcctgctccaagggcctcctgcatgagggcgcggtagagacccggacccgcgccgtgctcctgccgtttcgctgcgctccgcccgatttaaatggatcc

SEQ ID NO: 14 - DNA, 723 bp, Artificial Sequence
  Hybrid promoter 14b
accggtgctaaaagataggtcggggtaacccttcagatctggctcagctagcctgtctccaagatttaggactctgaatctctgtgggctcctccctgtccccactcccaaacgcctgacgcggtgccccctcgccctccgctgctcctttctaccgctttccctcctccctcccatgtcttttccgtccttggtctagggctctcggcctgcgcctctgcaaacaccccctcccctccaactccggcagaactccgaggggaggggccggaggccacccttcccgcctgtggtcagaggggggcagcgccgcagccccgggtttggggggcaggggccatctctgcgccccgcccgatcaggccactcggcgcactaggggtggagggcgggaagcgtgactcccagagaggggggtccggcttgggcaggtgcgggcactggcagggcccaggcgggctccgggggcgggcggttcaggttacagcccagcggggggcagggggcggcccgcggtttgggcgagttcgccagcctcgaaaggggccgggcgctatataacgggcgccgcggcggggagaagacgcagagcgctgctgggctgccgggtctcccgcttccccctcctgctccaagggcctcctgcatgagggcgcggtagagacccggacccgcgccgtgctcctgccgtttcgctgcgctccgcccgatttaaatggatcc

SEQ ID NO: 15 - DNA, 705 bp, Artificial Sequence
  Hybrid promoter 15a
accggtgctaaaagataggtcggggtaacccttcagatctggctcagctagcctgtctccaagatttaggactctgaatctctgtgggctcctccctgtccccactcccaaacgcctgacgcggtgccccctcgccctccgctgctcctttctaccgctttccctcctccctcccatgtcttttccgtccttggtctagggctctcggcctgcgcctctgcaaacaccccctcccctccaactccggcagaactccgaggggaggggccggaggccacccttcccgcctgtggtcagaggggggcagcgccgcagccccgggtttggggggcaggggccatctctgcgccccgcccgatcaggccactcggcgcactaggggtggagggcgggaagcgtgactcccagagaggggggtccggcttgggcaggtgcgggcactggcagggcccaggcgggctccgggggcgggcggttcaggttacagcccagcggggggcagggggcggcccgcggtttgccgagggtgggggagaaccgtatataagtgcagtagtcgccgtgaacgttctttttcgcagagcgctgctgtctcccgcttccccctcctgctccaagggcctcctgcatgagggcgcggtagagacccggacccgcgccgtgctcctgccgtttcgctgcgctccgcccgatttaaatggatcc

SEQ ID NO: 16 - DNA, 715 bp, Artificial Sequence
  Hybrid promoter 15b
accggtgctaaaagataggtcggggtaacccttcagatctggctcagctagcctgtctccaagatttaggactctgaatctctgtgggctcctccctgtccccactcccaaacgcctgacgcggtgccccctcgccctccgctgctcctttctaccgctttccctcctccctcccatgtcttttccgtccttggtctagggctctcggcctgcgcctctgcaaacaccccctcccctccaactccggcagaactccgaggggaggggccggaggccacccttcccgcctgtggtcagaggggggcagcgccgcagccccgggtttggggggcaggggccatctctgcgccccgcccgatcaggccactcggcgcactaggggtggagggcgggaagcgtgactcccagagaggggggtccggcttgggcaggtgcgggcactggcagggcccaggcgggctccgggggcgggcggttcaggttacagcccagcggggggcagggggcggcccgcggtttgccgagggtgggggagaaccgtatataagtgcagtagtcgccgtgaacgttctttttcgcagagcgctgctgggctgccgggtctcccgcttccccctcctgctccaagggcctcctgcatgagggcgcggtagagacccggacccgcgccgtgctcctgccgtttcgctgcgctccgcccgatttaaatggatcc

SEQ ID NO: 17 - DNA, 435 bp, Artificial Sequence
  Hybrid promoter 22a
accggtaccccctcccctccaactccggcagaactccgaggggaggggccggaggccacccttcccgcctgtggtcagaggggggcagcgccgcagccccgggtttggggggcaggggccatctctgcgccccgcccgatcaggccactcggcgcactaggggtggagggcgggaagcgtgactcccagagaggggggtccggcttgggcaggtgcgggcactggcagggcccaggcgggctccgggggcgggcggttcaggttacagcccagcggggggcagggggcggcccgcggtttgaccggtgcctagagaaggtggggcactggcagggcccaggcgggctccgggggcgggcgggtgagtcacccacacaaaggaaaagggcctttccgtcctcagccgtcgcttcatgtgactccacggagtaccgg

SEQ ID NO: 18 - DNA, 1437 bp, Artificial Sequence
  Hybrid promoter 1a
accggtgcctagagaaggtgaccccctcccctccaactccggcagaactccgaggggaggggccggaggccacccttcccgcctgtggtcagaggggggcagcgccgcagccccgggtttggggggcaggggccatctctgcgccccgcccgatcaggccactcggcgcactaggggtggagggcgggaagcgtgactcccagagaggggggtccggcttgggcaggtgcgggcactggcagggcccaggcgggctccgggggcgggcggttcaggttacagcccagcggggggcagggggcggcccgcggtttgccgagggtgggggagaaccgtatataagtgcagtagtcgccgtgaacgttctttttcgcaacgggtttgccgccagaacacaggtaagtgccgtgtgtggttcccgcgggcctggcctctttacgggttatggcccttgcgtgccttgaattacttccacctggctgcagtacgtgattcttgatcccgagcttcgggttggaagtgggtgggagagttcgaggccttgcgcttaaggagccccttcgcctcgtgcttgagttgaggcctggcctgggcgctggggccgccgcgtgcgaatctggtggcaccttcgcgcctgtctcgctgctttcgataagtctctagccatttaaaatttttgatgacctgctgcgacgctttttttctggcaagatagtcttgtaaatgcgggccaagatctgcacactggtatttcggtttttggggccgcgggcggcgacggggcccgtgcgtcccagcgcacatgttcggcgaggcggggcctgcgagcgcggccaccgagaatcggacgggggtagtctcaagctggccggcctgctctggtgcctggcctcgcgccgccgtgtatcgccccgccctgggcggcaaggctggcccggtcggcaccagttgcgtgagcggaaagatggccgcttcccggccctgctgcagggagctcaaaatggaggacgcggcgctcgggagagcgggcgggtgagtcacccacacaaaggaaaagggcctttccgtcctcagccgtcgcttcatgtgactccacggagtaccgggcgccgtccaggcacctcgattagttctcgagcttttggagtacgtcgtctttaggttggggggaggggttttatgcgatggagtttccccacactgagtgggtggagactgaagttaggccagcttggcacttgatgtaattctccttggaatttgccctttttgagtttggatcttggttcattctcaagcctcagacagtggttcaaagtttttttcttccatttcaggtgtcgtgaggaattagcttggtactaatacgactcactatagggagacccaagctggctaggtaagcttgatatcgaattcctgcagcccgggggatcc

SEQ ID NO: 19 - DNA, 1447 bp, Artificial Sequence
  Hybrid promoter 1b
accggtgcctagagaaggtgaccccctcccctccaactccggcagaactccgaggggaggggccggaggccacccttcccgcctgtggtcagaggggggcagcgccgcagccccgggtttggggggcaggggccatctctgcgccccgcccgatcaggccactcggcgcactaggggtggagggcgggaagcgtgactcccagagaggggggtccggcttgggcaggtgcgggcactggcagggcccaggcgggctccgggggcgggcggttcaggttacagcccagcggggggcagggggcggcccgcggtttgccgagggtgggggagaaccgtatataagtgcagtagtcgccgtgaacgttctttttcgcaacgggggctgccgggtttgccgccagaacacaggtaagtgccgtgtgtggttcccgcgggcctggcctctttacgggttatggcccttgcgtgccttgaattacttccacctggctgcagtacgtgattcttgatcccgagcttcgggttggaagtgggtgggagagttcgaggccttgcgcttaaggagccccttcgcctcgtgcttgagttgaggcctggcctgggcgctggggccgccgcgtgcgaatctggtggcaccttcgcgcctgtctcgctgctttcgataagtctctagccatttaaaatttttgatgacctgctgcgacgctttttttctggcaagatagtcttgtaaatgcgggccaagatctgcacactggtatttcggtttttggggccgcgggcggcgacggggcccgtgcgtcccagcgcacatgttcggcgaggcggggcctgcgagcgcggccaccgagaatcggacgggggtagtctcaagctggccggcctgctctggtgcctggcctcgcgccgccgtgtatcgccccgccctgggcggcaaggctggcccggtcggcaccagttgcgtgagcggaaagatggccgcttcccggccctgctgcagggagctcaaaatggaggacgcggcgctcgggagagcgggcgggtgagtcacccacacaaaggaaaagggcctttccgtcctcagccgtcgcttcatgtgactccacggagtaccgggcgccgtccaggcacctcgattagttctcgagcttttggagtacgtcgtctttaggttggggggaggggttttatgcgatggagtttccccacactgagtgggtggagactgaagttaggccagcttggcacttgatgtaattctccttggaatttgccctttttgagtttggatcttggttcattctcaagcctcagacagtggttcaaagtttttttcttccatttcaggtgtcgtgaggaattagcttggtactaatacgactcactatagggagacccaagctggctaggtaagcttgatatcgaattcctgcagcccgggggatcc

SEQ ID NO: 20 - DNA, 1182 bp, Artificial Sequence
  Hybrid promoter 5a
accggtgcctagagaaggtggggcactggcagggcccaggcgggctccgggggcgggcggccgagggtgggggagaaccgtatataagtgcagtagtcgccgtgaacgttctttttcgcaacgggtttgccgccagaacacaggtaagtgccgtgtgtggttcccgcgggcctggcctctttacgggttatggcccttgcgtgccttgaattacttccacctggctgcagtacgtgattcttgatcccgagcttcgggttggaagtgggtgggagagttcgaggccttgcgcttaaggagccccttcgcctcgtgcttgagttgaggcctggcctgggcgctggggccgccgcgtgcgaatctggtggcaccttcgcgcctgtctcgctgctttcgataagtctctagccatttaaaatttttgatgacctgctgcgacgctttttttctggcaagatagtcttgtaaatgcgggccaagatctgcacactggtatttcggtttttggggccgcgggcggcgacggggcccgtgcgtcccagcgcacatgttcggcgaggcggggcctgcgagcgcggccaccgagaatcggacgggggtagtctcaagctggccggcctgctctggtgcctggcctcgcgccgccgtgtatcgccccgccctgggcggcaaggctggcccggtcggcaccagttgcgtgagcggaaagatggccgcttcccggccctgctgcagggagctcaaaatggaggacgcggcgctcgggagagcgggcgggtgagtcacccacacaaaggaaaagggcctttccgtcctcagccgtcgcttcatgtgactccacggagtaccgggcgccgtccaggcacctcgattagttctcgagcttttggagtacgtcgtctttaggttggggggaggggttttatgcgatggagtttccccacactgagtgggtggagactgaagttaggccagcttggcacttgatgtaattctccttggaatttgccctttttgagtttggatcttggttcattctcaagcctcagacagtggttcaaagtttttttcttccatttcaggtgtcgtgaggaattagcttggtactaatacgactcactatagggagacccaagctggctaggtaagcttgatatcgaattcctgcagcccgggggatcc

SEQ ID NO: 21 - DNA, 1192 bp, Artificial Sequence
  Hybrid promoter 5b
accggtgcctagagaaggtggggcactggcagggcccaggcgggctccgggggcgggcggccgagggtgggggagaaccgtatataagtgcagtagtcgccgtgaacgttctttttcgcaacgggggctgccgggtttgccgccagaacacaggtaagtgccgtgtgtggttcccgcgggcctggcctctttacgggttatggcccttgcgtgccttgaattacttccacctggctgcagtacgtgattcttgatcccgagcttcgggttggaagtgggtgggagagttcgaggccttgcgcttaaggagccccttcgcctcgtgcttgagttgaggcctggcctgggcgctggggccgccgcgtgcgaatctggtggcaccttcgcgcctgtctcgctgctttcgataagtctctagccatttaaaatttttgatgacctgctgcgacgctttttttctggcaagatagtcttgtaaatgcgggccaagatctgcacactggtatttcggtttttggggccgcgggcggcgacggggcccgtgcgtcccagcgcacatgttcggcgaggcggggcctgcgagcgcggccaccgagaatcggacgggggtagtctcaagctggccggcctgctctggtgcctggcctcgcgccgccgtgtatcgccccgccctgggcggcaaggctggcccggtcggcaccagttgcgtgagcggaaagatggccgcttcccggccctgctgcagggagctcaaaatggaggacgcggcgctcgggagagcgggcgggtgagtcacccacacaaaggaaaagggcctttccgtcctcagccgtcgcttcatgtgactccacggagtaccgggcgccgtccaggcacctcgattagttctcgagcttttggagtacgtcgtctttaggttggggggaggggttttatgcgatggagtttccccacactgagtgggtggagactgaagttaggccagcttggcacttgatgtaattctccttggaatttgccctttttgagtttggatcttggttcattctcaagcctcagacagtggttcaaagtttttttcttccatttcaggtgtcgtgaggaattagcttggtactaatacgactcactatagggagacccaagctggctaggtaagcttgatatcgaattcctgcagcccgggggatcc

SEQ ID NO: 22 - DNA, 1205 bp, Artificial Sequence
  Hybrid promoter 11a
accggtgcctagagaaggtgaccccctccccgtgatgtcgtgcccaggcgggctccgggggcgggcggcccgcggtttgggcgccgagggtgggggagaaccgtatataagtgcagtagtcgccgtgaacgttctttttcgcaacgggtttgccgccagaacacaggtaagtgccgtgtgtggttcccgcgggcctggcctctttacgggttatggcccttgcgtgccttgaattacttccacctggctgcagtacgtgattcttgatcccgagcttcgggttggaagtgggtgggagagttcgaggccttgcgcttaaggagccccttcgcctcgtgcttgagttgaggcctggcctgggcgctggggccgccgcgtgcgaatctggtggcaccttcgcgcctgtctcgctgctttcgataagtctctagccatttaaaatttttgatgacctgctgcgacgctttttttctggcaagatagtcttgtaaatgcgggccaagatctgcacactggtatttcggtttttggggccgcgggcggcgacggggcccgtgcgtcccagcgcacatgttcggcgaggcggggcctgcgagcgcggccaccgagaatcggacgggggtagtctcaagctggccggcctgctctggtgcctggcctcgcgccgccgtgtatcgccccgccctgggcggcaaggctggcccggtcggcaccagttgcgtgagcggaaagatggccgcttcccggccctgctgcagggagctcaaaatggaggacgcggcgctcgggagagcgggcgggtgagtcacccacacaaaggaaaagggcctttccgtcctcagccgtcgcttcatgtgactccacggagtaccgggcgccgtccaggcacctcgattagttctcgagcttttggagtacgtcgtctttaggttggggggaggggttttatgcgatggagtttccccacactgagtgggtggagactgaagttaggccagcttggcacttgatgtaattctccttggaatttgccctttttgagtttggatcttggttcattctcaagcctcagacagtggttcaaagtttttttcttccatttcaggtgtcgtgaggaattagcttggtactaatacgactcactatagggagacccaagctggctaggtaagcttgatatcgaattcctgcagcccgggggatcc

SEQ ID NO: 23 - DNA, 1215 bp, Artificial Sequence
  Hybrid promoter 11b
accggtgcctagagaaggtgaccccctccccgtgatgtcgtgcccaggcgggctccgggggcgggcggcccgcggtttgggcgccgagggtgggggagaaccgtatataagtgcagtagtcgccgtgaacgttctttttcgcaacgggggctgccgggtttgccgccagaacacaggtaagtgccgtgtgtggttcccgcgggcctggcctctttacgggttatggcccttgcgtgccttgaattacttccacctggctgcagtacgtgattcttgatcccgagcttcgggttggaagtgggtgggagagttcgaggccttgcgcttaaggagccccttcgcctcgtgcttgagttgaggcctggcctgggcgctggggccgccgcgtgcgaatctggtggcaccttcgcgcctgtctcgctgctttcgataagtctctagccatttaaaatttttgatgacctgctgcgacgctttttttctggcaagatagtcttgtaaatgcgggccaagatctgcacactggtatttcggtttttggggccgcgggcggcgacggggcccgtgcgtcccagcgcacatgttcggcgaggcggggcctgcgagcgcggccaccgagaatcggacgggggtagtctcaagctggccggcctgctctggtgcctggcctcgcgccgccgtgtatcgccccgccctgggcggcaaggctggcccggtcggcaccagttgcgtgagcggaaagatggccgcttcccggccctgctgcagggagctcaaaatggaggacgcggcgctcgggagagcgggcgggtgagtcacccacacaaaggaaaagggcctttccgtcctcagccgtcgcttcatgtgactccacggagtaccgggcgccgtccaggcacctcgattagttctcgagcttttggagtacgtcgtctttaggttggggggaggggttttatgcgatggagtttccccacactgagtgggtggagactgaagttaggccagcttggcacttgatgtaattctccttggaatttgccctttttgagtttggatcttggttcattctcaagcctcagacagtggttcaaagtttttttcttccatttcaggtgtcgtgaggaattagcttggtactaatacgactcactatagggagacccaagctggctaggtaagcttgatatcgaattcctgcagcccgggggatcc

SEQ ID NO: 24 - DNA, 1200 bp, Artificial Sequence
  Hybrid promoter 12a
accggtgcctagagaaggtggcgcggggtaaactgggaaagtgatgcccaggcgtcgtgtactggctccgcctttttcccgagggtgggggagaaccgtatataagtgcagtagtcgccgtgaacgttctttttcgcaacgggtttgccgccagaacacaggtaagtgccgtgtgtggttcccgcgggcctggcctctttacgggttatggcccttgcgtgccttgaattacttccacctggctgcagtacgtgattcttgatcccgagcttcgggttggaagtgggtgggagagttcgaggccttgcgcttaaggagccccttcgcctcgtgcttgagttgaggcctggcctgggcgctggggccgccgcgtgcgaatctggtggcaccttcgcgcctgtctcgctgctttcgataagtctctagccatttaaaatttttgatgacctgctgcgacgctttttttctggcaagatagtcttgtaaatgcgggccaagatctgcacactggtatttcggtttttggggccgcgggcggcgacggggcccgtgcgtcccagcgcacatgttcggcgaggcggggcctgcgagcgcggccaccgagaatcggacgggggtagtctcaagctggccggcctgctctggtgcctggcctcgcgccgccgtgtatcgccccgccctgggcggcaaggctggcccggtcggcaccagttgcgtgagcggaaagatggccgcttcccggccctgctgcagggagctcaaaatggaggacgcggcgctcgggagagcgggcgggtgagtcacccacacaaaggaaaagggcctttccgtcctcagccgtcgcttcatgtgactccacggagtaccgggcgccgtccaggcacctcgattagttctcgagcttttggagtacgtcgtctttaggttggggggaggggttttatgcgatggagtttccccacactgagtgggtggagactgaagttaggccagcttggcacttgatgtaattctccttggaatttgccctttttgagtttggatcttggttcattctcaagcctcagacagtggttcaaagtttttttcttccatttcaggtgtcgtgaggaattagcttggtactaatacgactcactatagggagacccaagctggctaggtaagcttgatatcgaattcctgcagcccgggggatcc

SEQ ID NO: 25 - DNA, 1210 bp, Artificial Sequence
  Hybrid promoter 12b
accggtgcctagagaaggtggcgcggggtaaactgggaaagtgatgcccaggcgtcgtgtactggctccgcctttttcccgagggtgggggagaaccgtatataagtgcagtagtcgccgtgaacgttctttttcgcaacgggggctgccgggtttgccgccagaacacaggtaagtgccgtgtgtggttcccgcgggcctggcctctttacgggttatggcccttgcgtgccttgaattacttccacctggctgcagtacgtgattcttgatcccgagcttcgggttggaagtgggtgggagagttcgaggccttgcgcttaaggagccccttcgcctcgtgcttgagttgaggcctggcctgggcgctggggccgccgcgtgcgaatctggtggcaccttcgcgcctgtctcgctgctttcgataagtctctagccatttaaaatttttgatgacctgctgcgacgctttttttctggcaagatagtcttgtaaatgcgggccaagatctgcacactggtatttcggtttttggggccgcgggcggcgacggggcccgtgcgtcccagcgcacatgttcggcgaggcggggcctgcgagcgcggccaccgagaatcggacgggggtagtctcaagctggccggcctgctctggtgcctggcctcgcgccgccgtgtatcgccccgccctgggcggcaaggctggcccggtcggcaccagttgcgtgagcggaaagatggccgcttcccggccctgctgcagggagctcaaaatggaggacgcggcgctcgggagagcgggcgggtgagtcacccacacaaaggaaaagggcctttccgtcctcagccgtcgcttcatgtgactccacggagtaccgggcgccgtccaggcacctcgattagttctcgagcttttggagtacgtcgtctttaggttggggggaggggttttatgcgatggagtttccccacactgagtgggtggagactgaagttaggccagcttggcacttgatgtaattctccttggaatttgccctttttgagtttggatcttggttcattctcaagcctcagacagtggttcaaagtttttttcttccatttcaggtgtcgtgaggaattagcttggtactaatacgactcactatagggagacccaagctggctaggtaagcttgatatcgaattcctgcagcccgggggatcc

SEQ ID NO: 26 - DNA, 1214 bp, Artificial Sequence
  Hybrid promoter 23a
gaattggctccggtgcccgtcagtgggcagagcgcacatcgcccacagtccccgagaagttggggggaggggtcggcaattgaaccggtgggcactggcagggcccaggcgggctccgggggcgggcgggcctagagaaggtggggcactggcagggcccaggcgggctccgggggcgggcggccgagggtgggggagaaccgtatataagtgcagtagtcgccgtgaacgttctttttcgcaacgggtttgccgccagaacacaggtaagtgccgtgtgtggttcccgcgggcctggcctctttacgggttatggcccttgcgtgccttgaattacttccacctggctgcagtacgtgattcttgatcccgagcttcgggttggaagtgggtgggagagttcgaggccttgcgcttaaggagccccttcgcctcgtgcttgagttgaggcctggcctgggcgctggggccgccgcgtgcgaatctggtggcaccttcgcgcctgtctcgctgctttcgataagtctctagccatttaaaatttttgatgacctgctgcgacgctttttttctggcaagatagtcttgtaaatgcgggccaagatctgcacactggtatttcggtttttggggccgcgggcggcgacggggcccgtgcgtcccagcgcacatgttcggcgaggcggggcctgcgagcgcggccaccgagaatcggacgggggtagtctcaagctggccggcctgctctggtgcctggcctcgcgccgccgtgtatcgccccgccctgggcggcaaggctggcccggtcggcaccagttgcgtgagcggaaagatggccgcttcccggccctgctgcagggagctcaaaatggaggacgcggcgctcgggagagcgggcgggtgagtcacccacacaaaggaaaagggcctttccgtcctcagccgtcgcttcatgtgactccacggagtaccgggcgccgtccaggcacctcgattagttctcgagcttttggagtacgtcgtctttaggttggggggaggggttttatgcgatggagtttccccacactgagtgggtggagactgaagttaggccagcttggcacttgatgtaattctccttggaatttgccctttttgagtttggatcttggttcattctcaagcctcagacagtggttcaaagtttttttcttccatttcaggtgtcgtga

SEQ ID NO: 27 - DNA, 255 bp, Artificial Sequence
  Hybrid promoter 24a
gaattggctccggtgcccgtcagtgggcagagcgcacatcgcccacagtccccgagaagttggggggaggggtcggcaattgaaccggtgggcactggcagggcccaggcgggctccgggggcgggcgggggcactggcagggcccaggcgggctccgggggcgggcgggggcactggcagggcccaggcgggctccgggggcgggcgggggcactggcagggcccaggcgggctccgggggcgggcggaccggt

SEQ ID NO: 28 - DNA, 1556 bp, Artificial Sequence
  Hybrid promoter 25a
gaattggctccggtgcccgtcagtgggcagagcgcacatcgcccacagtccccgagaagttggggggaggggtcggcaattgaaccggtgcctagagaaggtgaccccctcccctccaactccggcagaactccgaggggaggggccggaggccacccttcccgcctgtggtcagaggggggcagcgccgcagccccgggtttggggggcaggggccatctctgcgccccgcccgatcaggccactcggcgcactaggggtggagggcgggaagcgtgactcccagagaggggggtccggcttgggcaggtgcgggcactggcagggcccaggcgggctccgggggcgggcggtgggcactggcagggcccaggcgggctccgggggcggtcaggttacagcccagcggggggcagggggcggcccgcggtttgccgagggtgggggagaaccgtatataagtgcagtagtcgccgtgaacgttctttttcgcaacgggtttgccgccagaacacaggtaagtgccgtgtgtggttcccgcgggcctggcctctttacgggttatggcccttgcgtgccttgaattacttccacctggctgcagtacgtgattcttgatcccgagcttcgggttggaagtgggtgggagagttcgaggccttgcgcttaaggagccccttcgcctcgtgcttgagttgaggcctggcctgggcgctggggccgccgcgtgcgaatctggtggcaccttcgcgcctgtctcgctgctttcgataagtctctagccatttaaaatttttgatgacctgctgcgacgctttttttctggcaagatagtcttgtaaatgcgggccaagatctgcacactggtatttcggtttttggggccgcgggcggcgacggggcccgtgcgtcccagcgcacatgttcggcgaggcggggcctgcgagcgcggccaccgagaatcggacgggggtagtctcaagctggccggcctgctctggtgcctggcctcgcgccgccgtgtatcgccccgccctgggcggcaaggctggcccggtcggcaccagttgcgtgagcggaaagatggccgcttcccggccctgctgcagggagctcaaaatggaggacgcggcgctcgggagagcgggcgggtgagtcacccacacaaaggaaaagggcctttccgtcctcagccgtcgcttcatgtgactccacggagtaccgggcgccgtccaggcacctcgattagttctcgagcttttggagtacgtcgtctttaggttggggggaggggttttatgcgatggagtttccccacactgagtgggtggagactgaagttaggccagcttggcacttgatgtaattctccttggaatttgccctttttgagtttggatcttggttcattctcaagcctcagacagtggttcaaagtttttttcttccatttcaggtgtcgtgaggaattagcttggtactaatacgactcactatagggagacccaagctggctaggtaagcttgatatcgaattcctgcagcccgggggatcc

SEQ ID NO: 29 - DNA, 1566 bp, Artificial Sequence
  Hybrid promoter 25b
gaattggctccggtgcccgtcagtgggcagagcgcacatcgcccacagtccccgagaagttggggggaggggtcggcaattgaaccggtgcctagagaaggtgaccccctcccctccaactccggcagaactccgaggggaggggccggaggccacccttcccgcctgtggtcagaggggggcagcgccgcagccccgggtttggggggcaggggccatctctgcgccccgcccgatcaggccactcggcgcactaggggtggagggcgggaagcgtgactcccagagaggggggtccggcttgggcaggtgcgggcactggcagggcccaggcgggctccgggggcgggcggtgggcactggcagggcccaggcgggctccgggggcggtcaggttacagcccagcggggggcagggggcggcccgcggtttgccgagggtgggggagaaccgtatataagtgcagtagtcgccgtgaacgttctttttcgcaacgggggctgccgggtttgccgccagaacacaggtaagtgccgtgtgtggttcccgcgggcctggcctctttacgggttatggcccttgcgtgccttgaattacttccacctggctgcagtacgtgattcttgatcccgagcttcgggttggaagtgggtgggagagttcgaggccttgcgcttaaggagccccttcgcctcgtgcttgagttgaggcctggcctgggcgctggggccgccgcgtgcgaatctggtggcaccttcgcgcctgtctcgctgctttcgataagtctctagccatttaaaatttttgatgacctgctgcgacgctttttttctggcaagatagtcttgtaaatgcgggccaagatctgcacactggtatttcggtttttggggccgcgggcggcgacggggcccgtgcgtcccagcgcacatgttcggcgaggcggggcctgcgagcgcggccaccgagaatcggacgggggtagtctcaagctggccggcctgctctggtgcctggcctcgcgccgccgtgtatcgccccgccctgggcggcaaggctggcccggtcggcaccagttgcgtgagcggaaagatggccgcttcccggccctgctgcagggagctcaaaatggaggacgcggcgctcgggagagcgggcgggtgagtcacccacacaaaggaaaagggcctttccgtcctcagccgtcgcttcatgtgactccacggagtaccgggcgccgtccaggcacctcgattagttctcgagcttttggagtacgtcgtctttaggttggggggaggggttttatgcgatggagtttccccacactgagtgggtggagactgaagttaggccagcttggcacttgatgtaattctccttggaatttgccctttttgagtttggatcttggttcattctcaagcctcagacagtggttcaaagtttttttcttccatttcaggtgtcgtgaggaattagcttggtactaatacgactcactatagggagacccaagctggctaggtaagcttgatatcgaattcctgcagcccgggggatcc

SEQ ID NO: 30 - DNA, 1224 bp, Artificial Sequence
  Hybrid promoter 23b
gaattggctccggtgcccgtcagtgggcagagcgcacatcgcccacagtccccgagaagttggggggaggggtcggcaattgaaccggtgggcactggcagggcccaggcgggctccgggggcgggcgggcctagagaaggtggggcactggcagggcccaggcgggctccgggggcgggcggccgagggtgggggagaaccgtatataagtgcagtagtcgccgtgaacgttctttttcgcaacgggggctgccgggtttgccgccagaacacaggtaagtgccgtgtgtggttcccgcgggcctggcctctttacgggttatggcccttgcgtgccttgaattacttccacctggctgcagtacgtgattcttgatcccgagcttcgggttggaagtgggtgggagagttcgaggccttgcgcttaaggagccccttcgcctcgtgcttgagttgaggcctggcctgggcgctggggccgccgcgtgcgaatctggtggcaccttcgcgcctgtctcgctgctttcgataagtctctagccatttaaaatttttgatgacctgctgcgacgctttttttctggcaagatagtcttgtaaatgcgggccaagatctgcacactggtatttcggtttttggggccgcgggcggcgacggggcccgtgcgtcccagcgcacatgttcggcgaggcggggcctgcgagcgcggccaccgagaatcggacgggggtagtctcaagctggccggcctgctctggtgcctggcctcgcgccgccgtgtatcgccccgccctgggcggcaaggctggcccggtcggcaccagttgcgtgagcggaaagatggccgcttcccggccctgctgcagggagctcaaaatggaggacgcggcgctcgggagagcgggcgggtgagtcacccacacaaaggaaaagggcctttccgtcctcagccgtcgcttcatgtgactccacggagtaccgggcgccgtccaggcacctcgattagttctcgagcttttggagtacgtcgtctttaggttggggggaggggttttatgcgatggagtttccccacactgagtgggtggagactgaagttaggccagcttggcacttgatgtaattctccttggaatttgccctttttgagtttggatcttggttcattctcaagcctcagacagtggttcaaagtttttttcttccatttcaggtgtcgtga